European Patent Application EP 4 458 373 A1, published November 6, 2024. Title: PROCESS FOR OBTAINING LIPOSOMAL PARTICLES COMPRISING AT LEAST ONE PNEUMOCOCCAL SURFACE PROTEIN A (PSPA) AND AN ADJUVANT MOLECULE FORMULATED IN NANOCOMPOSITE MICROPARTICLE CARRIERS (NCMP), LIPOSOMAL PARTICLES OBTAINED BY SAID PROCESS, USE THEREOF AND IMMUNOGENIC COMPOSITION. Applicant: INSTITUTO BUTANTAN. The sequence listing filed with the application follows.

SEQUENCE LISTING (4 sequences)

SEQ ID NO: 1 - protein, 326 aa, synthetic construct
  REGION 1..326: note = Purified PspA1
AMEEAPVASQSKAEKDYDAAVKKYEAAKKEYEDGKAAQKKYEDDQKKTEEKAEEERKASEEEQAANLKYQQELVKYIRENDPTKKAEAKKAMDEAEKEYKKKQTEFAEVRAKVIPSAEELKKTRQKAEEAKAKEAELTKKVEEAEKKVTEAKQKVDAEHAEEVAPQAKIAELEHEVQKLEKALKEIDESDSEDYVKEGLRAPLQFELDVKQAKLSKLEELSDKIDELDAEIAKLEKDVEDFKNSDGEQAGQYLAAAEEDLVAKKAELEKTEADLKKAVNEPEKPAEETPAPAPKPEQPAEQPKPAPAPQPEKPAEEPENPASAPQP

SEQ ID NO: 2 - DNA, 992 bp, synthetic construct
  misc_feature 1..992: note = purified PspA1 gene sequence
  source 1..992: mol_type = other DNA
tagccatggaagaagcgcccgtagctagycagtctaaagctgagaaagactatgatgcagcagtgaaaaaatatgaagctgctaagaaggaatatgaggacggaaaagctgctcagaaaaagtatgaagatgatcagaagaaaactgaggagaaagcggaagaagaaagaaaagcttctgaagaagaacaagctgcaaatctgaaatatcaacaagagttggttaaatatatacgtgaaaatgatccaacaaaaaaagctgaagctaagaaagcaatggatgaggctgagaaagagtataagaaaaaacaaacggaatttgctgaagttcgtgcaaaggtaattcctagcgcggaagaattaaaaaagactagacaaaaagcagaagaggctaaagcaaaagaagcagaacttactaaaaaagtagaagaagctgagaaaaaagttactgaagccaaacaaaaagtggatgcagaacatgctgaagaagtcgctcctcaagctaaaatcgctgaattggaacatgaagttcagaaactagaaaaagctctcaaagagattgatgagtctgattcagaagattatgttaaagaaggtctccgtgctcctcttcaatttgaattggatgttaagcaagctaaactatcaaaacttgaagagttgagtgataagattgatgagttagacgctgaaattgcaaaacttgaaaaagatgtagaagatttcaaaaactcagacggtgagcaagctggacaataccttgctgcagctgaagaagacttagttgctaaaaaagctgaattagaaaaaactgaagctgaccttaagaaagcagttaatgagccagaaaaaccagctgaagaaactccagctccagcaccaaaaccagagcaaccagctgaacaaccaaaaccagcgccggctcctcaaccagaaaaaccagctgaagagcctgagaatccagcttcagcaccacaaccataactcgagcta

SEQ ID NO: 3 - protein, 382 aa, synthetic construct
  REGION 1..382: note = purified PspA4Pro without His
MEEAPVASQSKAEKDYDAAMKKSEAAKKAYEEAKKKAEDAQKKYDEGQKKTEEKARKAEEASKEIAKATSEVQNAYVKYQRVQRNSRLNEKERKKQLAEIDEEINKAKQILNEKNEDFKKVREEVIPEPTELAKDQRKAEEAKAEEKVAKRKYDYATLKVALAKSKVEAEEAELDNKAENLQNKVADLEKEIANAEKTVADLEKEVAKLEKDVEDFKNSNGEQAEQYLAAAEKDLVAKKAELAEAKIKAATKKAELEKAEAELENLLSTLDPEGKTQDELDKEAAEAELNKKVEALQNQVAELEEELSKLEDNLKDAETNNVEDYIKEGLEEAIATKKAELEKTQKELDAALNELGPDGDEEETPAPAPQPEKPAPAPAPKP

SEQ ID NO: 4 - DNA, 1146 bp, synthetic construct
  misc_feature 1..1146: note = purified PspA4Pro gene sequence
  source 1..1146: mol_type = other DNA
atggaagaagcccccgtagctagtcagtctaaagctgagaaagactatgatgcagcaatgaaaaaatctgaagctgctaagaaggcttacgaagaagctaaaaagaaagcagaagacgctcagaagaaatatgacgagggtcagaagaaaactgaggaaaaagctcgtaaggcagaagaagcatcgaaggaaatagctaaagccacgtctgaggtccaaaatgcgtatgtaaagtatcagagagtccaacgtaatagtagactgaatgaaaaagaacgaaaaaaacaattagcagaaattgatgaagaaatcaataaagctaaacaaattttgaacgagaagaatgaagattttaaaaaagttagggaagaagtaattcctgaaccaactgagttagctaaggatcagagaaaagcagaagaggctaaagcagaagaaaaagtagctaagagaaaatatgattatgcaactctaaaggtagcactagcgaagagtaaagtagaagcagaagaagctgagttggataacaaagctgagaatcttcaaaataaagttgctgatttagaaaaagaaatagctaatgctgaaaaaacggtagcagatttagaaaaagaagttgctaaacttgaaaaagatgtagaagatttcaaaaactcaaacggtgagcaagctgaacaataccttgctgcagctgaaaaagacttagttgctaaaaaagctgaattagcagaagctaaaattaaagctgctactaaaaaagctgaattagaaaaagcagaagctgaacttgaaaacctattatctacactagaccctgaaggtaagactcaggatgaattagataaagaagctgctgaagctgagttgaataaaaaagttgaagctcttcaaaaccaagttgctgaattagaagaagaactttcaaaacttgaagataatcttaaagatgctgaaacaaacaacgttgaagactacattaaagaaggtttagaagaagctatcgcgactaaaaaagctgaattggaaaaaactcaaaaagaattagatgcagctcttaatgagttaggccctgatggagatgaagaagagactccagcgccagctcctcaaccagaaaaaccagctccagctccagcaccaaaacca